European Patent Specification EP 2 838 528 B1, published August 6, 2025. Title: Methods of Inhibition of SHC-1/p66 and Improving Motor Skills. Applicant: Industrial Technology Research Institute Chang, Shau-Feng Ma, Chun-Hsien Yang, Kuo-Yi. The sequence listing filed with the application follows.

SEQUENCE LISTING (4 sequences)

SEQ ID NO: 1 - DNA, 26 bp, Artificial Sequence
  SHC1 isoform p66 forward primer
cggaatgagtctctgtcatcgctgga

SEQ ID NO: 2 - DNA, 22 bp, artificial sequence
  SHC1 isoform p66 reverse primer
cgccgcctccactcagcttgtt

SEQ ID NO: 3 - DNA, 18 bp, artificial sequence
  GAPDH forward primer
gaaggtgaaggtcggagt

SEQ ID NO: 4 - DNA, 20 bp, artificial sequence
  GAPDH reverse primer
gaagatggtgatgggatttc